European Patent Application EP 4 725 499 A1, published April 15, 2026. Title: ANTÍGENO QUIMÉRICO MULTIBLANCO PARA LA INMUNOTERAPIA DE LA ENFERMEDAD DE ALZHEIMER. Applicant: Centro de Neurociencias de Cuba, CNEURO. Application CU 2023-0023, filed May 12, 2023. The sequence listing filed with the application follows.

SEQUENCE LISTING (10 sequences)

SEQ ID NO: 1 - protein, 238 aa, unidentified
MAEPRQEFEVMEDHAGTYGLGDRKDQGGYTMHQDQEGDTDAGLKESPLGGGGSDAEFRHDSGYEVGGGGSFNNFTVSFWLRVPKVSASHLEGGGGSKGAIIGLMVGGVVIAGGGGSSKCGSLGNIHHKPGGGQVEVKSEKLDFKDRVQSKIGSLDNITHVPGGGNKKIETHKLTFRENAKAKTDHGAEIVYKEPVVSGDTEPRHLSNVSSTGSIDMVDEPQLATLADEVSASLAKQGL

SEQ ID NO: 2 - protein, 308 aa, unidentified
MVDKRMALVELKVPDIGGHENVDIIAVEVNVGDTIAVDDTLITLDLDHDDDDDKASDLLAMAEPRQEFEVMEDHAGTYGLGDRKDQGGYTMHQDQEGDTDAGLKESPLGGGGSDAEFRHDSGYEVGGGGSFNNFTVSFWLRVPKVSASHLEGGGGSKGAIIGLMVGGVVIAGGGGSSKCGSLGNIHHKPGGGQVEVKSEKLDFKDRVQSKIGSLDNITHVPGGGNKKIETHKLTFRENAKAKTDHGAEIVYKEPVVSGDTEPRHLSNVSSTGSIDMVDEPQLATLADEVSASLAKQGLGSRAHHHHHH

SEQ ID NO: 3 - DNA, 727 bp, synthetic construct
  source 1..727: mol_type = other DNA
gctagccatggccgaaccgcgccaagaattcgaagtgatggaagatcacgccggcacctatggtctgggcgatcgcaaagatcaaggtggttataccatgcaccaagatcaagaaggtgataccgatgccggtttaaaagaaagtccgctgggtggtggcggtagtgatgccgaatttcgccatgacagcggctatgaagttggcggcggcggcagctttaacaatttcaccgttagcttttggctgcgcgtgccgaaggttagcgcaagccatctggaaggtggcggcggtagcaaaggtgccatcattggtctgatggtgggcggtgttgtgatcgctggtggtggtggtagcagcaaatgcggttctttaggcaacattcatcacaaaccgggtggcggtcaagttgaggtgaaaagcgagaagctggacttcaaggaccgcgttcagagcaaaatcggctctttagacaacattacccatgtgccgggcggcggcaacaagaaaattgagacccacaagctgacctttcgcgaaaacgcaaaggccaaaaccgatcacggtgccgagatcgtttacaaagagccggtggtgagtggtgataccgaaccgcgtcatttaagcaatgtgagcagcaccggcagcattgatatggttgatgaaccgcagctggccactttagcagatgaagtgagcgcctctttagccaaacaaggtctgggatcc

SEQ ID NO: 4 - DNA, 202 bp, synthetic construct
  source 1..202: mol_type = other DNA
gctagccggtggtggcggtagtgatgccgaatttcgccatgacagcggctatgaagttggcggcggcggcagctttaacaatttcaccgttagcttttggctgcgcgtgccgaaggttagcgcaagccatctggaaggtggcggcggtagcaaaggtgccatcattggtctgatggtgggcggtgttgtgatcgctggatcc

SEQ ID NO: 5 - DNA, 616 bp, synthetic construct
  source 1..616: mol_type = other DNA
gctagccatggccgaaccgcgccaagaatttgaggtgatggaggaccatgccggtacctatggtttaggtgatcgtaaggatcaaggtggctataccatgcatcaagatcaagaaggtgataccgatgctggtctgaaagaaagtccgctgggtggcggcggcagctttaacaactttaccgtgagcttttggctgcgtgtgccgaaagtgagcgccagccatctggaaggtggcggtggcagcagtaaatgcggctctttaggcaatattcaccataaaccgggcggtggtcaagttgaagtgaagagcgagaaactggacttcaaagaccgcgtgcagagcaaaatcggctctttagacaacattacccatgtgccgggtggcggcaacaagaaaattgagacccataaactgaccttccgcgaaaacgccaaagccaaaaccgatcatggcgccgagatcgtgtataaagaaccggtggtgagcggcgatacagaaccgcgtcatctgagcaatgttagcagcaccggcagcatcgatatggtggatgagcctcagctggccactttagccgacgaagttagcgcctctttagccaaacaaggtctgggatcc

SEQ ID NO: 6 - DNA, 924 bp, synthetic construct
  source 1..924: mol_type = other DNA
atggtagataaaagaatggctttagttgaattgaaagtgcccgacattggcggacacgaaaatgtagatattatcgcggttgaagtaaacgtgggcgacactattgctgtggacgataccctgattactttggatctagatcacgatgacgatgacgataaagcttcagatctgctagccatggccgaaccgcgccaagaattcgaagtgatggaagatcacgccggcacctatggtctgggcgatcgcaaagatcaaggtggttataccatgcaccaagatcaagaaggtgataccgatgccggtttaaaagaaagtccgctgggtggtggcggtagtgatgccgaatttcgccatgacagcggctatgaagttggcggcggcggcagctttaacaatttcaccgttagcttttggctgcgcgtgccgaaggttagcgcaagccatctggaaggtggcggcggtagcaaaggtgccatcattggtctgatggtgggcggtgttgtgatcgctggtggtggtggtagcagcaaatgcggttctttaggcaacattcatcacaaaccgggtggcggtcaagttgaggtgaaaagcgagaagctggacttcaaggaccgcgttcagagcaaaatcggctctttagacaacattacccatgtgccgggcggcggcaacaagaaaattgagacccacaagctgacctttcgcgaaaacgcaaaggccaaaaccgatcacggtgccgagatcgtttacaaagagccggtggtgagtggtgataccgaaccgcgtcatttaagcaatgtgagcagcaccggcagcattgatatggttgatgaaccgcagctggccactttagcagatgaagtgagcgcctctttagccaaacaaggtctgggatcccgggcacaccatcaccatcaccat

SEQ ID NO: 7 - DNA, 399 bp, synthetic construct
  source 1..399: mol_type = other DNA
atggtagataaaagaatggctttagttgaattgaaagtgcccgacattggcggacacgaaaatgtagatattatcgcggttgaagtaaacgtgggcgacactattgctgtggacgataccctgattactttggatctagatcacgatgacgatgacgataaagcttcagatctgctagccggtggtggcggtagtgatgccgaatttcgccatgacagcggctatgaagttggcggcggcggcagctttaacaatttcaccgttagcttttggctgcgcgtgccgaaggttagcgcaagccatctggaaggtggcggcggtagcaaaggtgccatcattggtctgatggtgggcggtgttgtgatcgctggatcccgggcacaccatcaccatcaccat

SEQ ID NO: 8 - DNA, 813 bp, synthetic construct
  source 1..813: mol_type = other DNA
atggtagataaaagaatggctttagttgaattgaaagtgcccgacattggcggacacgaaaatgtagatattatcgcggttgaagtaaacgtgggcgacactattgctgtggacgataccctgattactttggatctagatcacgatgacgatgacgataaagcttcagatctgctagccatggccgaaccgcgccaagaatttgaggtgatggaggaccatgccggtacctatggtttaggtgatcgtaaggatcaaggtggctataccatgcatcaagatcaagaaggtgataccgatgctggtctgaaagaaagtccgctgggtggcggcggcagctttaacaactttaccgtgagcttttggctgcgtgtgccgaaagtgagcgccagccatctggaaggtggcggtggcagcagtaaatgcggctctttaggcaatattcaccataaaccgggcggtggtcaagttgaagtgaagagcgagaaactggacttcaaagaccgcgtgcagagcaaaatcggctctttagacaacattacccatgtgccgggtggcggcaacaagaaaattgagacccataaactgaccttccgcgaaaacgccaaagccaaaaccgatcatggcgccgagatcgtgtataaagaaccggtggtgagcggcgatacagaaccgcgtcatctgagcaatgttagcagcaccggcagcatcgatatggtggatgagcctcagctggccactttagccgacgaagttagcgcctctttagccaaacaaggtctgggatcccgggcacaccatcaccatcaccat

SEQ ID NO: 9 - protein, 133 aa, unidentified
MVDKRMALVELKVPDIGGHENVDIIAVEVNVGDTIAVDDTLITLDLDHDDDDDKASDLLAGGGGSDAEFRHDSGYEVGGGGSFNNFTVSFWLRVPKVSASHLEGGGGSKGAIIGLMVGGVVIAGSRAHHHHHH

SEQ ID NO: 10 - protein, 271 aa, unidentified
MVDKRMALVELKVPDIGGHENVDIIAVEVNVGDTIAVDDTLITLDLDHDDDDDKASDLLAMAEPRQEFEVMEDHAGTYGLGDRKDQGGYTMHQDQEGDTDAGLKESPLGGGGSFNNFTVSFWLRVPKVSASHLEGGGGSSKCGSLGNIHHKPGGGQVEVKSEKLDFKDRVQSKIGSLDNITHVPGGGNKKIETHKLTFRENAKAKTDHGAEIVYKEPVVSGDTEPRHLSNVSSTGSIDMVDEPQLATLADEVSASLAKQGLGSRAHHHHHH